European Patent Application EP 4 219 711 A1, published August 2, 2023. Title: ANTISENSE COMPOUNDS FOR THE TREATMENT OF CORONAVIRUS INFECTION. Applicant: CEINGE BIOTECNOLOGIE AVANZATE SCARL Zollo, Massimo Ferrucci, Veronica De Antonellis, Pasqualino. The sequence listing filed with the application follows.

SEQUENCE LISTING (24 sequences)

SEQ ID NO: 1 - RNA, 23 nt, Unknown
  SARS-CoV-2
ucgaucucuuguagaucuguucu

SEQ ID NO: 2 - RNA, 10 nt, Unknown
  SARS-CoV-2
cuaaacgaac

SEQ ID NO: 3 - RNA, 16 nt, Unknown
  SARS-CoV-2
augucugauaauggac

SEQ ID NO: 4 - RNA, 16 nt, Unknown
  SARS-CoV-2
augucucuaaauggac

SEQ ID NO: 5 - RNA, 10 nt, Unknown
  SARS-CoV-2
cuaaacgaac

SEQ ID NO: 6 - RNA, 16 nt, Unknown
  SARS-CoV-2
augucugauaauggac

SEQ ID NO: 7 - DNA, 37 bp, Artificial Sequence
  antisense oligonucleotide
  misc_feature (2)..(2): T or U
  misc_feature (6)..(7): T or U
  misc_feature (9)..(9): T or U
  misc_feature (16)..(19): T or U
  misc_feature (22)..(24): T or U
  misc_feature (26)..(27): T or U
  misc_feature (30)..(32): T or U
gnccannancagacannnnagnnngnncgnnnagaga

SEQ ID NO: 8 - RNA, 37 nt, Artificial Sequence
  antisense oligonucleotide
guccauuaucagacauuuuaguuuguucguuuagaga

SEQ ID NO: 9 - DNA, 37 bp, Artificial Sequence
  antisense oligonucleotide
gtccattatcagacattttagtttgttcgtttagaga

SEQ ID NO: 10 - DNA, 37 bp, Artificial Sequence
  artificial oligonucleotide
tctctaaacgaacaaactaaaatgtctgataatggac

SEQ ID NO: 11 - DNA, 26 bp, Artificial Sequence
  oligonucleotide primer
acaggtacgttaatagttaatagcgt

SEQ ID NO: 12 - DNA, 22 bp, Artificial Sequence
  oligonucleotide primer
atattgcagcagtacgcacaca

SEQ ID NO: 13 - DNA, 22 bp, Artificial Sequence
  oligonucleotide primer
gaaattcccaaagaccagtgga

SEQ ID NO: 14 - DNA, 22 bp, Artificial Sequence
  oligonucleotide primer
ccccaactatctctcgcttcat

SEQ ID NO: 15 - DNA, 24 bp, Artificial Sequence
  oligonucleotide primer
gacccagatcatgtttgagacctt

SEQ ID NO: 16 - DNA, 21 bp, Artificial Sequence
  oligonucleotide primer
ccagaggcgtacagggatagc

SEQ ID NO: 17 - DNA, 23 bp, Artificial Sequence
  oligonucleotide primer
caaccaactttcgatctcttgta

SEQ ID NO: 18 - DNA, 20 bp, Artificial Sequence
  oligonucleotide primer
tctgctcccttctgcgtaga

SEQ ID NO: 19 - DNA, 25 bp, Artificial Sequence
  oligonucleotide probe
  modified_base (1)..(1): 5'FAM-A
  modified_base (25)..(25): A-BBQ3'
acttcctcaaggaacaacattgcca

SEQ ID NO: 20 - DNA, 23 bp, Artificial Sequence
  oligonucleotide primer
cgatctcttgtagatctgttctc

SEQ ID NO: 21 - DNA, 22 bp, Artificial Sequence
  oligonucleotide primer
atattgcagcagtacgcacaca

SEQ ID NO: 22 - DNA, 26 bp, Artificial Sequence
  oligonucleotide probe
  modified_base (1)..(1): 5'FAM-A
  modified_base (25)..(25): G-BBQ-3'
  modified_base (26)..(26): G-BBQ-3'
acactagccatccttactgcgcttcg

SEQ ID NO: 23 - DNA, 23 bp, Artificial Sequence
  oligonucleotide primer
caaccaactttcgatctcttgta

SEQ ID NO: 24 - DNA, 22 bp, Artificial Sequence
  oligonucleotide primer
tctggttactgccagttgaatc